European Patent Application EP 4 613 875 A1, published September 10, 2025. Title: 一种高效且快速进行核酸文库构建的方法. Applicant: 深圳华大智造科技股份有限公司. Application CN. The sequence listing filed with the application follows.

SEQUENCE LISTING (4 sequences)

SEQ ID NO: 1 - DNA, 25 bp, synthetic construct
  source 1..25: mol_type = other DNA
gaacgacatggctacgatccgactt

SEQ ID NO: 2 - DNA, 18 bp, synthetic construct
  source 1..18: mol_type = other DNA
aagtcggaggccaagcgg

SEQ ID NO: 3 - DNA, 17 bp, synthetic construct
  source 1..17: mol_type = other DNA
gaacgacatggctacga

SEQ ID NO: 4 - DNA, 59 bp, synthetic construct
  source 1..59: mol_type = other DNA
tgtgagccaaggagttgatcggacctattgtcttcctaagaccgcttggcctccgactt